European Patent Specification EP 4 106 872 B1, published July 15, 2026. Title: COMPOSITIONS AND METHODS FOR ASSESSING THE EFFICACY OF INHIBITORS OF NEUROTRANSMITTER TRANSPORTERS. Applicant: DENOVO BIOPHARMA LLC Whitaker, John W. Dhali, Zafrin Sun, Hong Lu, Haiping Li, Xiaojun Wu, Wilson Luo, Wen. The sequence listing filed with the application follows.

SEQUENCE LISTING (51 sequences)

SEQ ID NO: 1 - DNA, 201 bp, Homo sapiens
  allele (101)..(101): y is c or t
aaaataggacacaatttctttttagaagctcacctcatatcaagtacatattctaatgcaaagtatgaatttcacaaagggctgagtatgtaggtgttggygccactgttctgatgttagcacccagcacttatttttctaacttttagaaaaatgtttactaatttctgccagttgcacccctttgtagtcacctcccag

SEQ ID NO: 2 - DNA, 201 bp, Homo sapiens
  allele (101)..(101): k is t or g
tttaatctttttattttgataaagaactataaaatgggacatatggatatacatctaaagtctccaaatttccatagtgtgttttttgagcatctttttaktattattatactttaagttctgagatacatgtgcagaatgtgcaggttgttacataggtatacacgtgtcatggtggtttgctgcacccatcaacccgtc

SEQ ID NO: 3 - DNA, 201 bp, Homo sapiens
  allele (101)..(101): y is c or t
gtaggtgctaaggcataccacaaatgaataaagcaagatattccctgacttcacagttttataaacataggttaacaagtaattcttattactcacacatyctggtgagtgctatagtagaaaaatatattattggagtaccatattaggaaaaagcattttgtatatgactggccagtgaagaagcattgaatttatccc

SEQ ID NO: 4 - DNA, 201 bp, Homo sapiens
  allele (101)..(101): w is a or t
ttgaaaatatttcatcaatgtattattccacttgtatttcatatagttcagtcactttattcagtaagaaaggaactggcaggagtttgtagtcagggatwtcattcattgtagtggaacaaggtatgggggaagtggaagagatgtagtccaagaaatattctgaggattattatttacaatatattcctagttatagtt

SEQ ID NO: 5 - DNA, 201 bp, Homo sapiens
  allele (101)..(101): k is g or t
ttaaataaaaggattatatctctatggtggaatgtactgcaggcattaaatcaatgtttatgtacctctacacaaataaactagaaaatctagaagaaatkgataaattcctggacacatacaccctcccaagactaaaccaggaagaagtccaatccctgaatggaccaataacaagttctgaaattgaggcagtaatta

SEQ ID NO: 6 - DNA, 201 bp, Homo sapiens
  allele (101)..(101): s is c or g
accatgaagtgctcgctcacctccacggtcatagtgcaatattcctttgtttgtcgattataaggtgcacttcaaaccttccccaacatctccctccaggstccttttcttaatgtgcctacaattagtcagtcgtattttgccacctcacaactttaaacaaagttctacatttcagacacaagtggaaaaatgaggcca

SEQ ID NO: 7 - DNA, 201 bp, Homo sapiens
  misc_feature (101)..(101): allele: n is a or absent
tgtctccaaataaataggagccgtatttgggtctggaagccatgaagtcttggggagagcttcacagatgtttggtgggtttccaaagacaattagcatantactccaagagtggagtgaaatagaatgtgtgcttgtttcttttctttgttagtaccaaaatagatttgtgtttatttgatagaaaaaaaaaattctagc

SEQ ID NO: 8 - DNA, 201 bp, Homo sapiens
  allele (101)..(101): r is g or a
agagactcaaaataactcaaattctttggctacgaataactctatttatctgcaaaaagccacatgaaccctaattctttctaagcacaaagaaacagagragaggatatataaatagtagcaatcattggaacaaaagttgaaatgagggtagaaatagagactcccaccctctgttctcccttctaataggcacaaata

SEQ ID NO: 9 - DNA, 201 bp, Homo sapiens
  allele (101)..(101): y is c or t
acaaatattcatggaagaataagaaacttcagagcaacatgggtctctggacaagtcataatttttagaagtgagtggagacttagagggaacagtaagayaagaaaatagcagggaaagaccataaagtaacggacttgtctagttaataagcattttcctggaaatgaatggaataggatacaatggtgagaatacaca

SEQ ID NO: 10 - DNA, 201 bp, Homo sapiens
  allele (101)..(101): y is t or c
caattctcttaggattccccagggagatcccagcctgttaattttccccagtagttgtcagcaggcagggccagcagagctacgtgcattgttatcagctyagcctgtgaccaggcacgaaatggctgtgcttggcttgcgcatctccatatccacgtgcagtccatgatgtcatggaggccgtgttgcctcctgcacagc

SEQ ID NO: 11 - DNA, 201 bp, Homo sapiens
  allele (101)..(101): m is a or c
aagacctaaagcagaaacatcatttgacccagcaatcccattactgggtatatacccaaaggagtataaatcatccttttataaagacacatgcacacatmcgttctttgcagcaccagtcacaataacaaagacatggaatcaacctaaatgcccatcaatgatagaccgaataaagaaaatgtggtacatatacaccat

SEQ ID NO: 12 - DNA, 201 bp, Homo sapiens
  allele (101)..(101): m is a or c
aaccaggtggattcacagagaaaaactctgtctgaggaatttgggaaaggctttacccggggacattagagctggtcctggagagtagatagggtgggctmtcctggacatagatgacttgttctctgttcatccattggatattcccaagccgttttcttttgctaccctttccagcagaaatgccaactacttactttt

SEQ ID NO: 13 - DNA, 201 bp, Homo sapiens
  allele (101)..(101): s is g or c
ctggagagtagatagggtgggctatcctggacatagatgacttgttctctgttcatccattggatattcccaagccgttttcttttgctaccctttccagsagaaatgccaactacttacttttccagtctcccttgcagctggggttgcggcgggcgggcgggggaggggggcggggggcgcaatacaacatgcagttct

SEQ ID NO: 14 - DNA, 201 bp, Homo sapiens
  allele (101)..(101): s is g or c
aagtgggagctaaataaagagaacacataggcacagagaggggaacaacagacactggggccttttggagggtggagggtgggaggagagsgaggatctgsaaaaaccaccaatgggtactaggtttaatacctgggtgatgaaataatctgtataacaaacccccatgacacaagtttacatatataacacacctgcacg

SEQ ID NO: 15 - DNA, 201 bp, Homo sapiens
  allele (101)..(101): y is t or c
gcatataatgtcctttctaaatcccttttcttatagaaaaacatcgtaagtttttataaaaagataggattaatttatttttaagctaacaacaaaggtgytaccagcccactgtagttaaaaaagaggaaggagaagtgttttttttttttttttttttttttaactttaagagaaaacaggccgggctcagtggctcaa

SEQ ID NO: 16 - DNA, 201 bp, Homo sapiens
  allele (101)..(101): r is g or a
tatagaaaaacatcgtaagtttttataaaaagataggattaatttatttttaagctaacaacaaaggtgttaccagcccactgtagttaaaaaagaggaargagaagtgttttttttttttttttttttttttaactttaagagaaaacaggccgggctcagtggctcaagcctgtaatcccagcactttcggaggctgag

SEQ ID NO: 17 - DNA, 201 bp, Homo sapiens
  allele (101)..(101): r is g or a
ctaacaacaaaggtgttaccagcccactgtagttaaaaaagaggaaggagaagtgttttttttttttttttttttttttaactttaagagaaaacaggccrggctcagtggctcaagcctgtaatcccagcactttcggaggctgaggcgggcagatcactgaaggtcaggagttcctgaccagcctggccaacatggtga

SEQ ID NO: 18 - DNA, 201 bp, Homo sapiens
  allele (101)..(101): y is t or c
attttttaaaaatcgctatgaatagcattgaaaaattaatttaaaaagaaaaaatatataaaaatcactattcaaatattgctctcaaagtagaagaatgyattaaaacatgacactgttttgaaggccctatcatgaatccaacaaatacttacagcgcagtaaatgggagaacacaattataacatcacagttcttatc

SEQ ID NO: 19 - DNA, 201 bp, Homo sapiens
  allele (101)..(101): r is g or a
tcagcatttgtgagctagctctgaaaactcaagctaaacatcaacctgagataacatttcttactttgcaaacatactgttaatagttgaaagtaataggrgaaatcgggaggaaaggagggggcataacctaaataagtggaaaccaatccctgtgcattccattctcaatacaaggtatcaccacatattggttacaga

SEQ ID NO: 20 - DNA, 201 bp, Homo sapiens
  allele (101)..(101): y is c or t
tcacagatggaaggcaaggtcacggaaggcaagcaaggctgagatggttttagagacaggtggcatggaggatctctcccttgctttacaatttgccccaycacactccatgaattctaatatgctcttggagtgagggatatagccgtccttgttctagcactgaaagtggaatcctgggaaacctttcagtcctgggca

SEQ ID NO: 21 - DNA, 201 bp, Homo sapiens
  allele (101)..(101): r is a or g
atacccatgaaaatttgtcctctggatttgaacatgatcactgacatttcagtgatggaaaaacgtatgttgctatgtacattttctataccatgtccacrcagataacgtttctttaattcactcatttaacaaatatttattgggtaccttctttaatgaagcagcataatccaaacattatttaagacacccaaactc

SEQ ID NO: 22 - DNA, 201 bp, Homo sapiens
  allele (101)..(101): r is a or g
tggttgcagtgagctgagatcacaccactgcactccagtctgggtgacagagcaaggctctgtcccttggctccccactccctcccccaaaaaagaaaaaraaagctaaggacaaaaattcttaagtgacttccctttctcaagaaaaaaagaaaaaatctgttcttgttttataaaagtcccaggtacaagaattcctaa

SEQ ID NO: 23 - DNA, 201 bp, Homo sapiens
  allele (101)..(101): y is t or c
gtctggcctggagctactgaaaatcctgcctacaaggacttgtggaaggagcatcatgcctccgttattcccagaggccgagggaggaaaatgagcagacyagcctgtgtttttggaaggaaactcctaaaaactacaatcattcagaggcagcctggatcatctgcaaaacgtaaaaagaacctttaaattcctcttaaa

SEQ ID NO: 24 - DNA, 201 bp, Homo sapiens
  allele (101)..(101): r is g or a
ctttacccggggacattagagctggtcctggagagtagatagggtgggctatcctggacatagatgacttgttctctgttcatccattggatattcccaarccgttttcttttgctaccctttccagcagaaatgccaactacttacttttccagtctcccttgcagctggggttgcggcgggcgggcgggggaggggggc

SEQ ID NO: 25 - DNA, 201 bp, Homo sapiens
  allele (101)..(101): k is g or t
cctctgtgcccctctcaccaaccctgtagaagtaggaatagaaatgaattaagcagcaccacagtggactagagaagggcccagactccaggaccagactkcctggatatgaatcccagcatggtcacttactaggaaaataaccttagataagtgaccccatctgcctgtgcctcagtttccacatttctaaagtgtaga

SEQ ID NO: 26 - DNA, 201 bp, Homo sapiens
  allele (101)..(101): r is a or g
gaccccatctgcctgtgcctcagtttccacatttctaaagtgtagaaatgaggatatagaagaaagtactcatgagattttgaaatgaaagagtatttatraagtgcttaatccagtaagtactatataaaaataaggagtcaaatttaaaaaaattagaagacagccagggcaattaatcccagctgcatactgcctagt

SEQ ID NO: 27 - DNA, 201 bp, Homo sapiens
  allele (101)..(101): r is a or g
cctctcccatccaatctttatccctctccttcctttttcttctcctggcttttgacccagctaccaaggatccactgggggaactccaaggaactggtggrtaatggagccccaagctggaaggcgcttggtttccaaataactgcagcctctacaccaagccacattggactgtgacgtgaaccagaaacaaacttttat

SEQ ID NO: 28 - DNA, 201 bp, Homo sapiens
  allele (101)..(101): y is t or c
aatgggagaacacaattataacatcacagttcttatcacaaagattgccatagtctagatctgagaaggcttttaattagtatttctaacatttatcatgyccagtgaatgacagcttagacaaaaatcagtggcttcaacacttctcaaaattattcagtaattattctccaggtttctaattcatcagcttggtagatt

SEQ ID NO: 29 - DNA, 201 bp, Homo sapiens
  allele (101)..(101): y is c or t
gtgaggcataaggtaatgggaaatactacaatggaaaacacagacgatagaatattagagggaaaaagctttcacatctttataattctacactttaccgytgtttataaatgttgcagtatatccacaaatcagttaaattcatatatttcaaagccaaccaagagataaaactaaaagttaaagaggaagaaaaaaatt

SEQ ID NO: 30 - DNA, 201 bp, Homo sapiens
  allele (101)..(101): y is c or t
ttaccaattgtggcaacaactgtggatgtactacatcaatatattatgatctagacaatccacacatgaaatagtgtcaattctagttatctcatgatggytaagagaggatttaaggggtatcacgattctctgtcttatgaagaccagctaaagaaacagggagcgtttaacttgaagagaagcagcagcaccaacata

SEQ ID NO: 31 - DNA, 201 bp, Homo sapiens
  allele (101)..(101): m is a or c
ataaaaatagaggcatgatcagtagatttttttaaaaccagtatttattgtaaagcaatttgaaatcatgtttgtcatctccatcatatgaatttgagtamaaagtgatcctcttgcacatgcaatattttagttacataactttgtagcatcccccatcattttctaataaaacaatggtgggctttctctgactgggac

SEQ ID NO: 32 - DNA, 201 bp, Homo sapiens
  allele (101)..(101): r is g or a
aagtagtaatgttctttatgtctatttatgtccaatatctcatcgggtagaaggtggccaggccaggggcctcttgtgtggggagaagatttaaatgtccrtcccttggctaaggcagtataggcaggggaaagtcaaagttggaaataatcaaaataagaatgcaaatgaataagaaacaagatcctgggagttgaagag

SEQ ID NO: 33 - DNA, 201 bp, Homo sapiens
  allele (101)..(101): y is c or t
tttcattgtatactccacgtgttgcaataatgaaatacaagtagccctgtatcctagaattgtgtatctcactgcattgttcagtttattacaaccttgcytctgaaatttatttatcaagaagagcacattaactaaaagaagggaagagaaaatctctaggggcaatacatgatgctatacactagtgcatgtacacac

SEQ ID NO: 34 - DNA, 201 bp, Homo sapiens
  allele (101)..(101): y is c or t
tttctaagccttgatttcctcatcagcaaaatgcgaataatgtcaccttactcagagggttcatttaactgttatgtgagacaacaatgtttgacacctaycaattatttttatcgtaaattgaacctaacttttgctagcaggtttcctatcaatccaaactgaggtttgctagcaaagtctaaaagcatctgtttttgt

SEQ ID NO: 35 - DNA, 201 bp, Homo sapiens
  allele (101)..(101): m is  a or c
gtacatccatatgcaaaagaatgaagaatgaaactagactttcccttcttaccctacataaaaatcagctgaaaaggaatcagagacccaaatataagacmccaaatgataaaactactagaagaaaacacaggaaatactgtaggacattggtttgagaaaatattttatgactaagttctcaaaagcacaggcaaaaga

SEQ ID NO: 36 - DNA, 201 bp, Homo sapiens
  allele (101)..(101): m is a or c
aaggaatcagagacccaaatataagaccccaaatgataaaactactagaagaaaacacaggaaatactgtaggacattggtttgagaaaatattttatgamtaagttctcaaaagcacaggcaaaagaagcaaaaagaaacaaacttgattatatcaaactaaaaagcctctgcacagaaaaaaaaaataaaaaacaatca

SEQ ID NO: 37 - DNA, 201 bp, Homo sapiens
  allele (101)..(101): r is g or a
acagatttctgacctgtaactggaagaagttcttcatttactgagacaggcaagactatgggaagagcaggttgggcatgaagatcgtgagcttggtttgragcttgttatcattgagatgcccatttgacatctatctttggatatccccacaagcagaccttgagacacacatttgagtgcaagtaatctacccgggag

SEQ ID NO: 38 - DNA, 201 bp, Homo sapiens
  allele (101)..(101): y is c or t
ttgttttggttgaagtaggtcaaggataccagtcttcagggtactctagaagggtctcagggacacccaggggttcttgattgacctcatgatacaaaggyctaacacctccgaagagaacatttaagcaaaaggcaagactgagcaggaagcaaagtctaaataaatatagtgctactatttttgcaaagtacagatcag

SEQ ID NO: 39 - DNA, 201 bp, Homo sapiens
  allele (101)..(101): r is a or g
gacagcatagaacatttttatcaccactcagacttttactgggcagtgatgttctgtatcttcattccactggtggttccagggggtctcatttgttacartccatgaaaccgtacacttaaagctgagtgttttaagatatataaattacaccataatagaattgactacaaaaatggtttttgagagaaaattgtacca

SEQ ID NO: 40 - DNA, 201 bp, Homo sapiens
  allele (101)..(101): r is g or a
catttttatcaccactcagacttttactgggcagtgatgttctgtatcttcattccactggtggttccagggggtctcatttgttacaatccatgaaaccrtacacttaaagctgagtgttttaagatatataaattacaccataatagaattgactacaaaaatggtttttgagagaaaattgtaccaagaataaactgt

SEQ ID NO: 41 - DNA, 201 bp, Homo sapiens
  allele (101)..(101): r is g or a
tatatattatttccttgggcattccagattttgtcaaggaattttacattttgagaagttgtgcttgactgtcagcactttgctatgctatgataaaatcrgaggacaacaaaagtttgatttaagggcttggttaaaagtgttgaatttaagttacccctatctgtgagtcactatacttagggtgaccacacatcctgg

SEQ ID NO: 42 - DNA, 201 bp, Homo sapiens
  allele (101)..(101): r is g or a
acactatgttcatagggtgcttgtggaaattcaagtaaggtgaaatacatttcagggtagagagtgacaaaaagggaagctggagagctgggtggggcacrtgatggagtctttgtatattcaggtaggaaggctgcattgttcccgtgggcaagtgagggagctgctgaagggttttactgcgtaagtgacagagtcaga

SEQ ID NO: 43 - DNA, 201 bp, Homo sapiens
  allele (101)..(101): y is c or t
aggacccagggaccccatctcaggtattttatgacaggcaaaaacccaagggaattccagagcctgctgatatgaaagtcacatggttttgaagttatgaygctgaatctctgtaatccatcagatccaactatttgacaattgttgagtcacttataaataacacatcttgaggtgctttgttatcttctctcaagcagc

SEQ ID NO: 44 - DNA, 201 bp, Homo sapiens
  allele (101)..(101): r is a or g
taggagaaagtaagaaagaaaggaagtaaaagggacttatataaggagatgtggaataggaaagaaaggcaaggagaaaaagggggaaaagagggtacacrtattccaagtaaaataggtactcttaccccaaatagaatggatagaattttctctaaaaagcctttacagattagtaaagattaagagtttatttttgta

SEQ ID NO: 45 - DNA, 201 bp, Homo sapiens
  allele (101)..(101): m is a or c
ctaccattaattatccttggctaagacttagagccacagattactagttactaaaaagccacaaggaacaaaaattcattcattcttccattaacttattmatctatacagctgccaacaaatacctgctgagcatcttctatgtacaaaattattctgcttcacatgttattagcaatgtaaattttaactgacaaagac

SEQ ID NO: 46 - DNA, 201 bp, Homo sapiens
  allele (101)..(101): r is g or a
tagcctatttcttttttccctcctaagctgtaatggcatttgcacagctgttacaagggaagttttaaaaatgcaaataagaattaggtagactgcacaarctaataaagagagctttgccaaatattaaaaaacgttctcagtcaaaataatcatactaatgaaatagaaagctcatgtgggagtgattttcagtagttt

SEQ ID NO: 47 - DNA, 201 bp, Homo sapiens
  allele (101)..(101): m is a or c
atactgatgccatccaatcttcatgcacagagagtcaaagcaattttcccaaggtcaccaggttagttggtggctttgatgtagagctagactagaacccmgattttctgacaatgcactgaacagatgagattactcaagtatctgagaaggacacatttgagtaagcagttaaacaatgcacagttactagggagcatc

SEQ ID NO: 48 - DNA, 201 bp, Homo sapiens
  allele (101)..(101): k is g or t
tatgtatgatggtcatacctaattttctactctccaattcctaaattagctagtggttttaggaacacacctagcttaaacataactttcaatacaccagkttgctcttgcccaaagttttatatatatataaatatgtatgtatgtacatataaatacatatatatatatgtatgtatgtatgtattgaagagtgaggct

SEQ ID NO: 49 - DNA, 201 bp, Homo sapiens
  allele (101)..(101): w is a or t
aaatctgatctgcctgtggcaggcacagtgggtgggggagatagtcagaaagggaagaattgccatgagttgatgctctggagaaggtgaggctggcttawaaagtcttcactatccccatgcccggcttcacccaattcagatcaaactcttccataaacttccaggacacaccccaagctcagctaacttccctgaagc

SEQ ID NO: 50 - DNA, 201 bp, Homo sapiens
  allele (101)..(101): r is a or g
gttctcacttacaagtgggagctaaataaagagaacacataggcacagagaggggaacaacagacactggggccttttggagggtggagggtgggaggagrgagaggatctggaaaaaccaccaatgggtactaggtttaatacctgggtgatgaaataatctgtataacaaacccccatgacacaagtttacatatataa

SEQ ID NO: 51 - DNA, 201 bp, Homo sapiens
  allele (101)..(101): r is a or g
ttctttttgtcgcggtttaagcccattttctattgtgctaacctcagcaaaaaaggacatcagctagttaccattctcctcatgattaaaactaattaagrcatccttccatctctgtcattagaagcacatgcaaatgggcatgtttccttaatttctgattctaaattgagaaaagtataaagaagcaattctgggctt